European Patent Application EP 4 144 841 A1, published March 8, 2023. Title: Novel small RNA programmable endonuclease systems with improved PAM specificity and uses thereof. Applicant: Bayer AG. The sequence listing filed with the application follows.

SEQUENCE LISTING (30 sequences)

SEQ ID NO: 1 - protein, 1053 aa, other sequences
  RNA programmable DNA endonuclease
MKRNYILGLDIGITSVGYGIIDYETRDVIDAGVRLFKEANVENNEGRRSKRGARRLKRRRRHRIQRVKKLLFDYNLLTDHSELSGINPYEARVKGLSQKLSEEEFSAALLHLAKRRGVHNVNEVEEDTGNELSTKEQISRNSKALEEKYVAELQLERLKKDGEVRGSINRFKTSDYVKEAKQLLKVQKAYHQLDQSFIDTYIDLLETRRTYYEGPGEGSPFGWKDIKEWYEMLMGHCTYFPEELRSVKYAYNADLYNALNDLNNLVITRDENEKLEYYEKFQIIENVFKQKKKPTLKQIAKEILVNEEDIKGYRVTSTGKPEFTNLKVYHDIKDITARKEIIENAELLDQIAKILTIYQSSEDIQEELTNLNSELTQEEIEQISNLKGYTGTHNLSLKAINLILDELWHTNDNQIAIFNRLKLVPKKVDLSQQKEIPTTLVDDFILSPVVKRSFIQSIKVINAIIKKYGLPNDIIIELAREKNSKDAQKMINEMQKRNRQTNERIEEIIRTTGKENAKYLIEKIKLHDMQEGKCLYSLEAIPLEDLLNNPFNYEVDHIIPRSVSFDNSFNNKVLVKQEENSKKGNRTPFQYLSSSDSKISYETFKKHILNLAKGKGRISKTKKEYLLEERDINRFSVQKDFINRNLVDTRYATRGLMNLLRSYFRVNNLDVKVKSINGGFTSFLRRKWKFKKERNKGYKHHAEDALIIANADFIFKEWKKLDKAKKVMENQMFEEKQAESMPEIETEQEYKEIFITPHQIKHIKDFKDYKYSHRVDKKPNRELINDTLYSTRKDDKGNTLIVNNLNGLYDKDNDKLKKLINKSPEKLLMYHHDPQTYQKLKLIMEQYGDEKNPLYKYYEETGNYLTKYSKKDNGPVIKKIKYYGNKLNAHLDITDDYPNSRNKVVKLSLKPYRFDVYLDNGVYKFVTVKNLDVIKKENYYEVNSKCYEEAKKLKKISNQAEFIASFYNNDLIKINGELYRVIGVNNDLLNMIEVNMIDITYREYLENMNDKREPRIKKTIASKTQSIKKYSTDILGNLYEVKSKKHPQIIKKG

SEQ ID NO: 2 - protein, 1053 aa, other sequences
  RNA programmable DNA endonuclease
MKRNYILGLDIGITSVGYGIIDYETRDVIDAGVRLFKEANVENNEGRRSKRGARRLKRRRRHRIQRVKKLLFDYNLLTDHSELSGINPYEARVKGLSQKLSEEEFSAALLHLAKRRGVHNVNEVEEDTGNELSTKEQISRNSKALEEKYVAELQLERLKKDGEVRGSINRFKTSDYVKEAKQLLKVQKAYHQLDQSFIDTYIDLLETRRTYYEGPGEGSPFGWKDIKEWYEMLMGHCTYFPEELRSVKYAYNADLYNALNDLNNLVITRDENEKLEYYEKFQIIENVFKQKKKPTLKQIAKEILVNEEDIKGYRVTSTGKPEFTNLKVYHDIKDITARKEIIENAELLDQIAKILTIYQSSEDIQEELTNLNSELTQEEIEQISNLKGYTGTHNLSLKAINLILDELWHTNDNQIAIFNRLKLVPKKVDLSQQKEIPTTLVDDFILSPVVKRSFIQSIKVINAIIKKYGLPNDIIIELAREKNSKDAQKMINEMQKRNRQTNERIEEIIRTTGKENAKYLIEKIKLHDMQEGKCLYSLEAIPLEDLLNNPFNYEVDHIIPRSVSFDNSFNNKVLVKQEENSKKGNRTPFQYLSSSDSKISYETFKKHILNLAKGKGRISKTKKEYLLEERDINRFSVQKDFINRNLVDTRYATRGLMNLLRSYFRVNNLDVKVKSINGGFTSFLRRKWKFKKERNKGYKHHAEDALIIANADFIFKEWKKLDKAKKVMENQMFEEKQAESMPEIETEQEYKEIFITPHQIKHIKDFKDYKYSHRVDKKPNRELINDTLYSTRKDDKGNTLIVNNLNGLYDKDNDKLKKLINKSPEKLLMYHHDPQTYQKLKLIMEQYGDEKNPLYKYYEETGNYLTKYSKKDNGPVIKKIKYYGNKLNAHLDITDDYPNSRNKVVKLSLKPYRFDVYLDNGVYKFVTVKNLDVIKKENYYEVNSKCYEEAKKLKKISNQAEFIASFYNNDLIKINGELYRVIGVNNDLRNMIEVNMIDITYREYLENMNDKREPRIKKTIASKTQSIKKYSTDILGNLYEVKSKKHPQIIKKG

SEQ ID NO: 3 - protein, 1053 aa, other sequences
  RNA programmable DNA endonuclease
MKRNYILGLDIGITSVGYGIIDYETRDVIDAGVRLFKEANVENNEGRRSKRGARRLKRRRRHRIQRVKKLLFDYNLLTDHSELSGINPYEARVKGLSQKLSEEEFSAALLHLAKRRGVHNVNEVEEDTGNELSTKEQISRNSKALEEKYVAELQLERLKKDGEVRGSINRFKTSDYVKEAKQLLKVQKAYHQLDQSFIDTYIDLLETRRTYYEGPGEGSPFGWKDIKEWYEMLMGHCTYFPEELRSVKYAYNADLYNALNDLNNLVITRDENEKLEYYEKFQIIENVFKQKKKPTLKQIAKEILVNEEDIKGYRVTSTGKPEFTNLKVYHDIKDITARKEIIENAELLDQIAKILTIYQSSEDIQEELTNLNSELTQEEIEQISNLKGYTGTHNLSLKAINLILDELWHTNDNQIAIFNRLKLVPKKVDLSQQKEIPTTLVDDFILSPVVKRSFIQSIKVINAIIKKYGLPNDIIIELAREKNSKDAQKMINEMQKRNRQTNERIEEIIRTTGKENAKYLIEKIKLHDMQEGKCLYSLEAIPLEDLLNNPFNYEVDHIIPRSVSFDNSFNNKVLVKQEENSKKGNRTPFQYLSSSDSKISYETFKKHILNLAKGKGRISKTKKEYLLEERDINRFSVQKDFINRNLVDTRYATRGLMNLLRSYFRVNNLDVKVKSINGGFTSFLRRKWKFKKERNKGYKHHAEDALIIANADFIFKEWKKLDKAKKVMENQMFEEKQAESMPEIETEQEYKEIFITPHQIKHIKDFKDYKYSHRVDKKPNRELINDTLYSTRKDDKGNTLIVNNLNGLYDKDNDKLKKLINKSPEKLLMYHHDPQTYQKLKLIMEQYGDEKNPLYKYYEETGNYLTKYSKKDNGPVIKKIKYYGNKLNAHLDITDDYPNSRNKVVKLSLKPYRFDVYLDNGVYKFVTVKNLDVIKKENYYEVNSKCYEEAKKLKKISNQAEFIASFYNNDLIKINGELYRVIGVNNDLRNMIEVNMIDITYREYCENMNIKGEPRIKKTIASKTQSIKKYSTDILGNLYEVKSKKHPQIIKKG

SEQ ID NO: 4 - protein, 1053 aa, other sequences
  RNA programmable DNA endonuclease
MKRNYILGLDIGITSVGYGIIDYETRDVIDAGVRLFKEANVENNEGRRSKRGARRLKRRRRHRIQRVKKLLFDYNLLTDHSELSGINPYEARVKGLSQKLSEEEFSAALLHLAKRRGVHNVNEVEEDTGNELSTKEQISRNSKALEEKYVAELQLERLKKDGEVRGSINRFKTSDYVKEAKQLLKVQKAYHQLDQSFIDTYIDLLETRRTYYEGPGEGSPFGWKDIKEWYEMLMGHCTYFPEELRSVKYAYNADLYNALNDLNNLVITRDENEKLEYYEKFQIIENVFKQKKKPTLKQIAKEILVNEEDIKGYRVTSTGKPEFTNLKVYHDIKDITARKEIIENAELLDQIAKILTIYQSSEDIQEELTNLNSELTQEEIEQISNLKGYTGTHNLSLKAINLILDELWHTNDNQIAIFNRLKLVPKKVDLSQQKEIPTTLVDDFILSPVVKRSFIQSIKVINAIIKKYGLPNDIIIELAREKNSKDAQKMINEMQKRNRQTNERIEEIIRTTGKENAKYLIEKIKLHDMQEGKCLYSLEAIPLEDLLNNPFNYEVDHIIPRSVSFDNSFNNKVLVKQEENSKKGNRTPFQYLSSSDSKISYETFKKHILNLAKGKGRISKTKKEYLLEERDINRFSVQKDFINRNLVDTRYATRGLMNLLRSYFRVNNLDVKVKSINGGFTSFLRRKWKFKKERNKGYKHHAEDALIIANADFIFKEWKKLDKAKKVMENQMFEEKQAESMPEIETEQEYKEIFITPHQIKHIKDFKDYKYSHRVDKKPNRELINDTLYSTRKDDKGNTLIVNNLNGLYDKDNDKLKKLINKSPEKLLMYHHDPQTYQKLKLIMEQYGDEKNPLYKYYEETGNYLTKYSKKDNGPVIKKIKYYGNKLNAHLDITDDYPNSRNKVVKLSLKPYRFDVYLDNGVYKFVTVKNLDVIKKENYYEVNSKCYEEAKKLKKISNQAEFIASFYNNDLIKINGELYRVIGVNSDTRNMIEVNMIDITYREYLENMNDKREPRIKKTIASKTQSIKKYSTDILGNLYEVKSKKHPQIIKKG

SEQ ID NO: 5 - protein, 1053 aa, other sequences
  RNA programmable DNA endonuclease
MKRNYILGLDIGITSVGYGIIDYETRDVIDAGVRLFKEANVENNEGRRSKRGARRLKRRRRHRIQRVKKLLFDYNLLTDHSELSGINPYEARVKGLSQKLSEEEFSAALLHLAKRRGVHNVNEVEEDTGNELSTKEQISRNSKALEEKYVAELQLERLKKDGEVRGSINRFKTSDYVKEAKQLLKVQKAYHQLDQSFIDTYIDLLETRRTYYEGPGEGSPFGWKDIKEWYEMLMGHCTYFPEELRSVKYAYNADLYNALNDLNNLVITRDENEKLEYYEKFQIIENVFKQKKKPTLKQIAKEILVNEEDIKGYRVTSTGKPEFTNLKVYHDIKDITARKEIIENAELLDQIAKILTIYQSSEDIQEELTNLNSELTQEEIEQISNLKGYTGTHNLSLKAINLILDELWHTNDNQIAIFNRLKLVPKKVDLSQQKEIPTTLVDDFILSPVVKRSFIQSIKVINAIIKKYGLPNDIIIELAREKNSKDAQKMINEMQKRNRQTNERIEEIIRTTGKENAKYLIEKIKLHDMQEGKCLYSLEAIPLEDLLNNPFNYEVDHIIPRSVSFDNSFNNKVLVKQEENSKKGNRTPFQYLSSSDSKISYETFKKHILNLAKGKGRISKTKKEYLLEERDINRFSVQKDFINRNLVDTRYATRGLMNLLRSYFRVNNLDVKVKSINGGFTSFLRRKWKFKKERNKGYKHHAEDALIIANADFIFKEWKKLDKAKKVMENQMFEEKQAESMPEIETEQEYKEIFITPHQIKHIKDFKDYKYSHRVDKKPNRELINDTLYSTRKDDKGNTLIVNNLNGLYDKDNDKLKKLINKSPEKLLMYHHDPQTYQKLKLIMEQYGDEKNPLYKYYEETGNYLTKYSKKDNGPVIKKIKYYGNKLNAHLDITDDYPNSRNKVVKLSLKPYRFDVYLDNGVYKFVTVKNLDVIKKENYYEVNSKCYEEAKKLKKISNQAEFIASFYNNDLIKINGELYRVIGVNSDTRNMIEVNMIDITYREYCENMNIKGEPRIKKTIASKTQSIKKYSTDILGNLYEVKSKKHPQIIKKG

SEQ ID NO: 6 - protein, 1055 aa, other sequences
  RNA programmable DNA endonuclease
MKRNYILGLDIGITSVGYGIIDYETRDVIDAGVRLFKEANVENNEGRRSKRGARRLKRRRRHRIQRVKKLLFDYNLLTDHSELSGINPYEARVKGLSQKLSEEEFSAALLHLAKRRGVHNVNEVEEDTGNELSTKEQISRNSKALEEKYVAELQLERLKKDGEVRGSINRFKTSDYVKEAKQLLKVQKAYHQLDQSFIDTYIDLLETRRTYYEGPGEGSPFGWKDIKEWYEMLMGHCTYFPEELRSVKYAYNADLYNALNDLNNLVITRDENEKLEYYEKFQIIENVFKQKKKPTLKQIAKEILVNEEDIKGYRVTSTGKPEFTNLKVYHDIKDITARKEIIENAELLDQIAKILTIYQSSEDIQEELTNLNSELTQEEIEQISNLKGYTGTHNLSLKAINLILDELWHTNDNQIAIFNRLKLVPKKVDLSQQKEIPTTLVDDFILSPVVKRSFIQSIKVINAIIKKYGLPNDIIIELAREKNSKDAQKMINEMQKRNRQTNERIEEIIRTTGKENAKYLIEKIKLHDMQEGKCLYSLEAIPLEDLLNNPFNYEVDHIIPRSVSFDNSFNNKVLVKQEENSKKGNRTPFQYLSSSDSKISYETFKKHILNLAKGKGRISKTKKEYLLEERDINRFSVQKDFINRNLVDTRYATRGLMNLLRSYFRVNNLDVKVKSINGGFTSFLRRKWKFKKERNKGYKHHAEDALIIANADFIFKEWKKLDKAKKVMENQMFEEKQAESMPEIETEQEYKEIFITPHQIKHIKDFKDYKYSHRVDKKPNRELINDTLYSTRKDDKGNTLIVNNLNGLYDKDNDKLKKLINKSPEKLLMYHHDPQTYQKLKLIMEQYGDEKNPLYKYYEETGNYLTKYSKKDNGPVIKKIKYYGNKLNAHLDITDDYPNSRNKVVKLSIKPYRFDVYLTDKGYKFITISYLDVLKKDNYYYIPEQKYDKLKLGKAIDKNAKFIASFYKNDLIKLDGEIYKIIGVNSDTRNMIELDLPDIRYKEYCELNNIKGEPRIKKTIGKKVNSIEKLTTDVLGNVFTNTQYTKPQLLFKRGN

SEQ ID NO: 7 - protein, 1377 aa, other sequences
  protein sequence of full construct cloned into plasmid comprising NLS, nuclease, CLS, T2A-GFP used in Example
MKRPAATKKAGQAKKKKGGGGSGGGGSGGGGSGSMKRNYILGLDIGITSVGYGIIDYETRDVIDAGVRLFKEANVENNEGRRSKRGARRLKRRRRHRIQRVKKLLFDYNLLTDHSELSGINPYEARVKGLSQKLSEEEFSAALLHLAKRRGVHNVNEVEEDTGNELSTKEQISRNSKALEEKYVAELQLERLKKDGEVRGSINRFKTSDYVKEAKQLLKVQKAYHQLDQSFIDTYIDLLETRRTYYEGPGEGSPFGWKDIKEWYEMLMGHCTYFPEELRSVKYAYNADLYNALNDLNNLVITRDENEKLEYYEKFQIIENVFKQKKKPTLKQIAKEILVNEEDIKGYRVTSTGKPEFTNLKVYHDIKDITARKEIIENAELLDQIAKILTIYQSSEDIQEELTNLNSELTQEEIEQISNLKGYTGTHNLSLKAINLILDELWHTNDNQIAIFNRLKLVPKKVDLSQQKEIPTTLVDDFILSPVVKRSFIQSIKVINAIIKKYGLPNDIIIELAREKNSKDAQKMINEMQKRNRQTNERIEEIIRTTGKENAKYLIEKIKLHDMQEGKCLYSLEAIPLEDLLNNPFNYEVDHIIPRSVSFDNSFNNKVLVKQEENSKKGNRTPFQYLSSSDSKISYETFKKHILNLAKGKGRISKTKKEYLLEERDINRFSVQKDFINRNLVDTRYATRGLMNLLRSYFRVNNLDVKVKSINGGFTSFLRRKWKFKKERNKGYKHHAEDALIIANADFIFKEWKKLDKAKKVMENQMFEEKQAESMPEIETEQEYKEIFITPHQIKHIKDFKDYKYSHRVDKKPNRELINDTLYSTRKDDKGNTLIVNNLNGLYDKDNDKLKKLINKSPEKLLMYHHDPQTYQKLKLIMEQYGDEKNPLYKYYEETGNYLTKYSKKDNGPVIKKIKYYGNKLNAHLDITDDYPNSRNKVVKLSLKPYRFDVYLDNGVYKFVTVKNLDVIKKENYYEVNSKCYEEAKKLKKISNQAEFIASFYNNDLIKINGELYRVIGVNNDLLNMIEVNMIDITYREYLENMNDKREPRIKKTIASKTQSIKKYSTDILGNLYEVKSKKHPQIIKKGGGSGGSGGSGPPKKKRKVGGGGGSHHHHHHGGEGRGSLLTCGDVEENPGPEFMSGGEELFAGIVPVLIELDGDVHGHKFSVRGEGEGDADYGKLEIKFICTTGKLPVPWPTLVTTLCYGIQCFARYPEHMKMNDFFKSAMPEGYIQERTIQFQDDGKYKTRGEVKFEGDTLVNRIELKGKDFKEDGNILGHKLEYSFNSHNVYIRPDKANNGLEANFKTRHNIEGGGVQLADHYQTNVPLGDGPVLIPINHYLSTQTKISKDRNEARDHMVLLESFSACCHTHGMDELYR

SEQ ID NO: 8 - protein, 1377 aa, other sequences
  protein sequence of full construct cloned into plasmid comprising NLS, nuclease, CLS, T2A-GFP used in Example
MKRPAATKKAGQAKKKKGGGGSGGGGSGGGGSGSMKRNYILGLDIGITSVGYGIIDYETRDVIDAGVRLFKEANVENNEGRRSKRGARRLKRRRRHRIQRVKKLLFDYNLLTDHSELSGINPYEARVKGLSQKLSEEEFSAALLHLAKRRGVHNVNEVEEDTGNELSTKEQISRNSKALEEKYVAELQLERLKKDGEVRGSINRFKTSDYVKEAKQLLKVQKAYHQLDQSFIDTYIDLLETRRTYYEGPGEGSPFGWKDIKEWYEMLMGHCTYFPEELRSVKYAYNADLYNALNDLNNLVITRDENEKLEYYEKFQIIENVFKQKKKPTLKQIAKEILVNEEDIKGYRVTSTGKPEFTNLKVYHDIKDITARKEIIENAELLDQIAKILTIYQSSEDIQEELTNLNSELTQEEIEQISNLKGYTGTHNLSLKAINLILDELWHTNDNQIAIFNRLKLVPKKVDLSQQKEIPTTLVDDFILSPVVKRSFIQSIKVINAIIKKYGLPNDIIIELAREKNSKDAQKMINEMQKRNRQTNERIEEIIRTTGKENAKYLIEKIKLHDMQEGKCLYSLEAIPLEDLLNNPFNYEVDHIIPRSVSFDNSFNNKVLVKQEENSKKGNRTPFQYLSSSDSKISYETFKKHILNLAKGKGRISKTKKEYLLEERDINRFSVQKDFINRNLVDTRYATRGLMNLLRSYFRVNNLDVKVKSINGGFTSFLRRKWKFKKERNKGYKHHAEDALIIANADFIFKEWKKLDKAKKVMENQMFEEKQAESMPEIETEQEYKEIFITPHQIKHIKDFKDYKYSHRVDKKPNRELINDTLYSTRKDDKGNTLIVNNLNGLYDKDNDKLKKLINKSPEKLLMYHHDPQTYQKLKLIMEQYGDEKNPLYKYYEETGNYLTKYSKKDNGPVIKKIKYYGNKLNAHLDITDDYPNSRNKVVKLSLKPYRFDVYLDNGVYKFVTVKNLDVIKKENYYEVNSKCYEEAKKLKKISNQAEFIASFYNNDLIKINGELYRVIGVNNDLRNMIEVNMIDITYREYLENMNDKREPRIKKTIASKTQSIKKYSTDILGNLYEVKSKKHPQIIKKGGGSGGSGGSGPPKKKRKVGGGGGSHHHHHHGGEGRGSLLTCGDVEENPGPEFMSGGEELFAGIVPVLIELDGDVHGHKFSVRGEGEGDADYGKLEIKFICTTGKLPVPWPTLVTTLCYGIQCFARYPEHMKMNDFFKSAMPEGYIQERTIQFQDDGKYKTRGEVKFEGDTLVNRIELKGKDFKEDGNILGHKLEYSFNSHNVYIRPDKANNGLEANFKTRHNIEGGGVQLADHYQTNVPLGDGPVLIPINHYLSTQTKISKDRNEARDHMVLLESFSACCHTHGMDELYR

SEQ ID NO: 9 - protein, 1377 aa, other sequences
  protein sequence of full construct cloned into plasmid comprising NLS, nuclease, CLS, T2A-GFP used in Example
MKRPAATKKAGQAKKKKGGGGSGGGGSGGGGSGSMKRNYILGLDIGITSVGYGIIDYETRDVIDAGVRLFKEANVENNEGRRSKRGARRLKRRRRHRIQRVKKLLFDYNLLTDHSELSGINPYEARVKGLSQKLSEEEFSAALLHLAKRRGVHNVNEVEEDTGNELSTKEQISRNSKALEEKYVAELQLERLKKDGEVRGSINRFKTSDYVKEAKQLLKVQKAYHQLDQSFIDTYIDLLETRRTYYEGPGEGSPFGWKDIKEWYEMLMGHCTYFPEELRSVKYAYNADLYNALNDLNNLVITRDENEKLEYYEKFQIIENVFKQKKKPTLKQIAKEILVNEEDIKGYRVTSTGKPEFTNLKVYHDIKDITARKEIIENAELLDQIAKILTIYQSSEDIQEELTNLNSELTQEEIEQISNLKGYTGTHNLSLKAINLILDELWHTNDNQIAIFNRLKLVPKKVDLSQQKEIPTTLVDDFILSPVVKRSFIQSIKVINAIIKKYGLPNDIIIELAREKNSKDAQKMINEMQKRNRQTNERIEEIIRTTGKENAKYLIEKIKLHDMQEGKCLYSLEAIPLEDLLNNPFNYEVDHIIPRSVSFDNSFNNKVLVKQEENSKKGNRTPFQYLSSSDSKISYETFKKHILNLAKGKGRISKTKKEYLLEERDINRFSVQKDFINRNLVDTRYATRGLMNLLRSYFRVNNLDVKVKSINGGFTSFLRRKWKFKKERNKGYKHHAEDALIIANADFIFKEWKKLDKAKKVMENQMFEEKQAESMPEIETEQEYKEIFITPHQIKHIKDFKDYKYSHRVDKKPNRELINDTLYSTRKDDKGNTLIVNNLNGLYDKDNDKLKKLINKSPEKLLMYHHDPQTYQKLKLIMEQYGDEKNPLYKYYEETGNYLTKYSKKDNGPVIKKIKYYGNKLNAHLDITDDYPNSRNKVVKLSLKPYRFDVYLDNGVYKFVTVKNLDVIKKENYYEVNSKCYEEAKKLKKISNQAEFIASFYNNDLIKINGELYRVIGVNNDLRNMIEVNMIDITYREYCENMNIKGEPRIKKTIASKTQSIKKYSTDILGNLYEVKSKKHPQIIKKGGGSGGSGGSGPPKKKRKVGGGGGSHHHHHHGGEGRGSLLTCGDVEENPGPEFMSGGEELFAGIVPVLIELDGDVHGHKFSVRGEGEGDADYGKLEIKFICTTGKLPVPWPTLVTTLCYGIQCFARYPEHMKMNDFFKSAMPEGYIQERTIQFQDDGKYKTRGEVKFEGDTLVNRIELKGKDFKEDGNILGHKLEYSFNSHNVYIRPDKANNGLEANFKTRHNIEGGGVQLADHYQTNVPLGDGPVLIPINHYLSTQTKISKDRNEARDHMVLLESFSACCHTHGMDELYR

SEQ ID NO: 10 - protein, 1377 aa, other sequences
  protein sequence of full construct cloned into plasmid comprising NLS, nuclease, CLS, T2A-GFP used in Example
MKRPAATKKAGQAKKKKGGGGSGGGGSGGGGSGSMKRNYILGLDIGITSVGYGIIDYETRDVIDAGVRLFKEANVENNEGRRSKRGARRLKRRRRHRIQRVKKLLFDYNLLTDHSELSGINPYEARVKGLSQKLSEEEFSAALLHLAKRRGVHNVNEVEEDTGNELSTKEQISRNSKALEEKYVAELQLERLKKDGEVRGSINRFKTSDYVKEAKQLLKVQKAYHQLDQSFIDTYIDLLETRRTYYEGPGEGSPFGWKDIKEWYEMLMGHCTYFPEELRSVKYAYNADLYNALNDLNNLVITRDENEKLEYYEKFQIIENVFKQKKKPTLKQIAKEILVNEEDIKGYRVTSTGKPEFTNLKVYHDIKDITARKEIIENAELLDQIAKILTIYQSSEDIQEELTNLNSELTQEEIEQISNLKGYTGTHNLSLKAINLILDELWHTNDNQIAIFNRLKLVPKKVDLSQQKEIPTTLVDDFILSPVVKRSFIQSIKVINAIIKKYGLPNDIIIELAREKNSKDAQKMINEMQKRNRQTNERIEEIIRTTGKENAKYLIEKIKLHDMQEGKCLYSLEAIPLEDLLNNPFNYEVDHIIPRSVSFDNSFNNKVLVKQEENSKKGNRTPFQYLSSSDSKISYETFKKHILNLAKGKGRISKTKKEYLLEERDINRFSVQKDFINRNLVDTRYATRGLMNLLRSYFRVNNLDVKVKSINGGFTSFLRRKWKFKKERNKGYKHHAEDALIIANADFIFKEWKKLDKAKKVMENQMFEEKQAESMPEIETEQEYKEIFITPHQIKHIKDFKDYKYSHRVDKKPNRELINDTLYSTRKDDKGNTLIVNNLNGLYDKDNDKLKKLINKSPEKLLMYHHDPQTYQKLKLIMEQYGDEKNPLYKYYEETGNYLTKYSKKDNGPVIKKIKYYGNKLNAHLDITDDYPNSRNKVVKLSLKPYRFDVYLDNGVYKFVTVKNLDVIKKENYYEVNSKCYEEAKKLKKISNQAEFIASFYNNDLIKINGELYRVIGVNSDTRNMIEVNMIDITYREYLENMNDKREPRIKKTIASKTQSIKKYSTDILGNLYEVKSKKHPQIIKKGGGSGGSGGSGPPKKKRKVGGGGGSHHHHHHGGEGRGSLLTCGDVEENPGPEFMSGGEELFAGIVPVLIELDGDVHGHKFSVRGEGEGDADYGKLEIKFICTTGKLPVPWPTLVTTLCYGIQCFARYPEHMKMNDFFKSAMPEGYIQERTIQFQDDGKYKTRGEVKFEGDTLVNRIELKGKDFKEDGNILGHKLEYSFNSHNVYIRPDKANNGLEANFKTRHNIEGGGVQLADHYQTNVPLGDGPVLIPINHYLSTQTKISKDRNEARDHMVLLESFSACCHTHGMDELYR

SEQ ID NO: 11 - protein, 1377 aa, other sequences
  protein sequence of full construct cloned into plasmid comprising NLS, nuclease, CLS, T2A-GFP used in Example
MKRPAATKKAGQAKKKKGGGGSGGGGSGGGGSGSMKRNYILGLDIGITSVGYGIIDYETRDVIDAGVRLFKEANVENNEGRRSKRGARRLKRRRRHRIQRVKKLLFDYNLLTDHSELSGINPYEARVKGLSQKLSEEEFSAALLHLAKRRGVHNVNEVEEDTGNELSTKEQISRNSKALEEKYVAELQLERLKKDGEVRGSINRFKTSDYVKEAKQLLKVQKAYHQLDQSFIDTYIDLLETRRTYYEGPGEGSPFGWKDIKEWYEMLMGHCTYFPEELRSVKYAYNADLYNALNDLNNLVITRDENEKLEYYEKFQIIENVFKQKKKPTLKQIAKEILVNEEDIKGYRVTSTGKPEFTNLKVYHDIKDITARKEIIENAELLDQIAKILTIYQSSEDIQEELTNLNSELTQEEIEQISNLKGYTGTHNLSLKAINLILDELWHTNDNQIAIFNRLKLVPKKVDLSQQKEIPTTLVDDFILSPVVKRSFIQSIKVINAIIKKYGLPNDIIIELAREKNSKDAQKMINEMQKRNRQTNERIEEIIRTTGKENAKYLIEKIKLHDMQEGKCLYSLEAIPLEDLLNNPFNYEVDHIIPRSVSFDNSFNNKVLVKQEENSKKGNRTPFQYLSSSDSKISYETFKKHILNLAKGKGRISKTKKEYLLEERDINRFSVQKDFINRNLVDTRYATRGLMNLLRSYFRVNNLDVKVKSINGGFTSFLRRKWKFKKERNKGYKHHAEDALIIANADFIFKEWKKLDKAKKVMENQMFEEKQAESMPEIETEQEYKEIFITPHQIKHIKDFKDYKYSHRVDKKPNRELINDTLYSTRKDDKGNTLIVNNLNGLYDKDNDKLKKLINKSPEKLLMYHHDPQTYQKLKLIMEQYGDEKNPLYKYYEETGNYLTKYSKKDNGPVIKKIKYYGNKLNAHLDITDDYPNSRNKVVKLSLKPYRFDVYLDNGVYKFVTVKNLDVIKKENYYEVNSKCYEEAKKLKKISNQAEFIASFYNNDLIKINGELYRVIGVNSDTRNMIEVNMIDITYREYCENMNIKGEPRIKKTIASKTQSIKKYSTDILGNLYEVKSKKHPQIIKKGGGSGGSGGSGPPKKKRKVGGGGGSHHHHHHGGEGRGSLLTCGDVEENPGPEFMSGGEELFAGIVPVLIELDGDVHGHKFSVRGEGEGDADYGKLEIKFICTTGKLPVPWPTLVTTLCYGIQCFARYPEHMKMNDFFKSAMPEGYIQERTIQFQDDGKYKTRGEVKFEGDTLVNRIELKGKDFKEDGNILGHKLEYSFNSHNVYIRPDKANNGLEANFKTRHNIEGGGVQLADHYQTNVPLGDGPVLIPINHYLSTQTKISKDRNEARDHMVLLESFSACCHTHGMDELYR

SEQ ID NO: 12 - protein, 1379 aa, other sequences
  protein sequence of full construct cloned into plasmid comprising NLS, nuclease, CLS, T2A-GFP used in Example
MKRPAATKKAGQAKKKKGGGGSGGGGSGGGGSGSMKRNYILGLDIGITSVGYGIIDYETRDVIDAGVRLFKEANVENNEGRRSKRGARRLKRRRRHRIQRVKKLLFDYNLLTDHSELSGINPYEARVKGLSQKLSEEEFSAALLHLAKRRGVHNVNEVEEDTGNELSTKEQISRNSKALEEKYVAELQLERLKKDGEVRGSINRFKTSDYVKEAKQLLKVQKAYHQLDQSFIDTYIDLLETRRTYYEGPGEGSPFGWKDIKEWYEMLMGHCTYFPEELRSVKYAYNADLYNALNDLNNLVITRDENEKLEYYEKFQIIENVFKQKKKPTLKQIAKEILVNEEDIKGYRVTSTGKPEFTNLKVYHDIKDITARKEIIENAELLDQIAKILTIYQSSEDIQEELTNLNSELTQEEIEQISNLKGYTGTHNLSLKAINLILDELWHTNDNQIAIFNRLKLVPKKVDLSQQKEIPTTLVDDFILSPVVKRSFIQSIKVINAIIKKYGLPNDIIIELAREKNSKDAQKMINEMQKRNRQTNERIEEIIRTTGKENAKYLIEKIKLHDMQEGKCLYSLEAIPLEDLLNNPFNYEVDHIIPRSVSFDNSFNNKVLVKQEENSKKGNRTPFQYLSSSDSKISYETFKKHILNLAKGKGRISKTKKEYLLEERDINRFSVQKDFINRNLVDTRYATRGLMNLLRSYFRVNNLDVKVKSINGGFTSFLRRKWKFKKERNKGYKHHAEDALIIANADFIFKEWKKLDKAKKVMENQMFEEKQAESMPEIETEQEYKEIFITPHQIKHIKDFKDYKYSHRVDKKPNRELINDTLYSTRKDDKGNTLIVNNLNGLYDKDNDKLKKLINKSPEKLLMYHHDPQTYQKLKLIMEQYGDEKNPLYKYYEETGNYLTKYSKKDNGPVIKKIKYYGNKLNAHLDITDDYPNSRNKVVKLSIKPYRFDVYLTDKGYKFITISYLDVLKKDNYYYIPEQKYDKLKLGKAIDKNAKFIASFYKNDLIKLDGEIYKIIGVNSDTRNMIELDLPDIRYKEYCELNNIKGEPRIKKTIGKKVNSIEKLTTDVLGNVFTNTQYTKPQLLFKRGNGGSGGSGGSGPPKKKRKVGGGGGSHHHHHHGGEGRGSLLTCGDVEENPGPEFMSGGEELFAGIVPVLIELDGDVHGHKFSVRGEGEGDADYGKLEIKFICTTGKLPVPWPTLVTTLCYGIQCFARYPEHMKMNDFFKSAMPEGYIQERTIQFQDDGKYKTRGEVKFEGDTLVNRIELKGKDFKEDGNILGHKLEYSFNSHNVYIRPDKANNGLEANFKTRHNIEGGGVQLADHYQTNVPLGDGPVLIPINHYLSTQTKISKDRNEARDHMVLLESFSACCHTHGMDELYR

SEQ ID NO: 13 - DNA, 21 bp, other sequences
  NNGG guide
caaacagctacatatttggga

SEQ ID NO: 14 - DNA, 21 bp, other sequences
  NNGG guide
cccaaatatgtagctgtttgg

SEQ ID NO: 15 - DNA, 21 bp, other sequences
  NNGG guide
agctgtttgggaggtcagaaa

SEQ ID NO: 16 - DNA, 21 bp, other sequences
  NNGG guide
agagggaatgggctttggaaa

SEQ ID NO: 17 - DNA, 21 bp, other sequences
  NNGG guide
ctagggggcgctcggccacca

SEQ ID NO: 18 - DNA, 21 bp, other sequences
  NNGG guide
ccgccgccggccggggaggag

SEQ ID NO: 19 - DNA, 21 bp, other sequences
  NNGG guide
ggccggcggcggacagtggac

SEQ ID NO: 20 - DNA, 21 bp, other sequences
  NNGG guide
gcggcgagccgcgggcagggg

SEQ ID NO: 21 - DNA, 21 bp, other sequences
  NNGG guide
ggaggcggggtggagggggtc

SEQ ID NO: 22 - DNA, 21 bp, other sequences
  NNGG guide
gaagcgagaacagcccagaag

SEQ ID NO: 23 - DNA, 21 bp, other sequences
  NNGRRT guide
gctgtttgggaggtcagaaat

SEQ ID NO: 24 - DNA, 21 bp, other sequences
  NNGRRT guide
ccattccctctttagccagag

SEQ ID NO: 25 - DNA, 21 bp, other sequences
  NNGRRT guide
gcgctcggccaccacagggaa

SEQ ID NO: 26 - DNA, 21 bp, other sequences
  NNGRRT guide
gaatggagcgagcagcgtctt

SEQ ID NO: 27 - DNA, 21 bp, other sequences
  NNGRRT guide
tgccctgtggggcaaggtgaa

SEQ ID NO: 28 - DNA, 21 bp, other sequences
  NNGRRT guide
cagtaacggcagacttctcct

SEQ ID NO: 29 - DNA, 21 bp, other sequences
  NNGRRT guide
ctgactaccaagcatcgggca

SEQ ID NO: 30 - DNA, 21 bp, other sequences
  NNGRRT guide
gtgtgagggagcaccgttctc